European Patent Specification EP 4 120 958 B1, published April 29, 2026. Title: IMPLANTABLE CELL CHAMBER DEVICE AND USES THEREOF. Applicant: MILLENNIUM PHARMACEUTICALS, INC. The sequence listing filed with the application follows.

SEQUENCE LISTING (52 sequences)

SEQ ID NO: 1 - protein, 121 aa, Artificial Sequence [sequence omitted]

SEQ ID NO: 2 - protein, 5 aa, Artificial Sequence
  Description of Artificial Sequence: Synthetic peptide
SYWMH

SEQ ID NO: 3 - protein, 17 aa, Artificial Sequence
  Description of Artificial Sequence: Synthetic peptide
EIDPSESNTNYNQKFKG

SEQ ID NO: 4 - protein, 12 aa, Artificial Sequence
  Description of Artificial Sequence: Synthetic peptide
GGYDGWDYAIDY

SEQ ID NO: 5 - protein, 112 aa, Artificial Sequence [sequence omitted]

SEQ ID NO: 6 - protein, 16 aa, Artificial Sequence
  Description of Artificial Sequence: Synthetic peptide
RSSQSLAKSYGNTYLS

SEQ ID NO: 7 - protein, 7 aa, Artificial Sequence
  Description of Artificial Sequence: Synthetic peptide
GISNRFS

SEQ ID NO: 8 - protein, 9 aa, Artificial Sequence
  Description of Artificial Sequence: Synthetic peptide
LQGTHQPYT

SEQ ID NO: 9 - protein, 451 aa, Artificial Sequence
  Description of Artificial Sequence: Synthetic polypeptide
QVQLVQSGAEVKKPGASVKVSCKGSGYTFTSYWMHWVRQAPGQRLEWIGEIDPSESNTNYNQKFKGRVTLTVDISASTAYMELSSLRSEDTAVYYCARGGYDGWDYAIDYWGQGTLVTVSSASTKGPSVFPLAPSSKSTSGGTAALGCLVKDYFPEPVTVSWNSGALTSGVHTFPAVLQSSGLYSLSSVVTVPSSSLGTQTYICNVNHKPSNTKVDKKVEPKSCDKTHTCPPCPAPELAGAPSVFLFPPKPKDTLMISRTPEVTCVVVDVSHEDPEVKFNWYVDGVEVHNAKTKPREEQYNSTYRVVSVLTVLHQDWLNGKEYKCKVSNKALPAPIEKTISKAKGQPREPQVYTLPPSRDELTKNQVSLTCLVKGFYPSDIAVEWESNGQPENNYKTTPPVLDSDGSFFLYSKLTVDKSRWQQGNVFSCSVMHEALHNHYTQKSLSLSPGK

SEQ ID NO: 10 - protein, 219 aa, Artificial Sequence
  Description of Artificial Sequence: Synthetic polypeptide
DVVMTQSPLSLPVTPGEPASISCRSSQSLAKSYGNTYLSWYLQKPGQSPQLLIYGISNRFSGVPDRFSGSGSGTDFTLKISRVEAEDVGVYYCLQGTHQPYTFGQGTKVEIKRTVAAPSVFIFPPSDEQLKSGTASVVCLLNNFYPREAKVQWKVDNALQSGNSQESVTEQDSKDSTYSLSSTLTLSKADYEKHKVYACEVTHQGLSSPVTKSFNRGEC

SEQ ID NO: 11 - DNA, 336 bp, Artificial Sequence
  Description of Artificial Sequence: Synthetic polynucleotide
gatgtagtgatgactcaaagtccactctccctgcctgtcacccctggagaaccagcttctatctcttgcaggtctagtcagagtcttgcaaagagttatgggaacacctatttgtcttggtacctgcagaagcctggccagtctccacagctcctcatctatgggatttccaacagattttctggggtgccagacaggttcagtggcagtggttcagggacagatttcacactcaagatctcgcgagtagaggctgaggacgtgggagtgtattactgcttacaaggtacacatcagccgtacacgttcggacaggggaccaaggtggagatcaag

SEQ ID NO: 12 - DNA, 363 bp, Artificial Sequence
  Description of Artificial Sequence: Synthetic polynucleotide
caggtgcaattggtgcagtctggggctgaggttaagaagcctggggcttcagtgaaggtgtcctgcaagggttctggctacaccttcaccagctactggatgcattgggtgaggcaggcgcctggccaacgtctagagtggatcggagagattgatccttctgagagtaatactaactacaatcaaaaattcaagggacgcgtcacattgactgtagacatttccgctagcacagcctacatggagctctccagcctgagatctgaggacactgcggtctactattgtgcaagagggggttacgacggatgggactatgctattgactactggggtcaaggcaccctggtcaccgtcagctca

SEQ ID NO: 13 - DNA, 657 bp, Artificial Sequence
  Description of Artificial Sequence: Synthetic polynucleotide
gatgtagtgatgactcaaagtccactctccctgcctgtcacccctggagaaccagcttctatctcttgcaggtctagtcagagtcttgcaaagagttatgggaacacctatttgtcttggtacctgcagaagcctggccagtctccacagctcctcatctatgggatttccaacagattttctggggtgccagacaggttcagtggcagtggttcagggacagatttcacactcaagatctcgcgagtagaggctgaggacgtgggagtgtattactgcttacaaggtacacatcagccgtacacgttcggacaggggaccaaggtggagatcaagcgtacggtggctgcaccatctgtcttcatcttcccgccatctgatgagcagttgaaatctggaactgcctctgttgtgtgcctgctgaataacttctatcccagagaggccaaagtacagtggaaggtggataacgccctccaatcgggtaactcccaggagagtgtcacagagcaggacagcaaggacagcacctacagcctcagcagcaccctgaccctgagcaaagcagactacgagaaacacaaagtctacgcctgcgaagtcacccatcagggcctgagctcgcccgtcacaaagagcttcaacaggggagagtgt

SEQ ID NO: 14 - DNA, 1353 bp, Artificial Sequence
  Description of Artificial Sequence: Synthetic polynucleotide
caggtgcaattggtgcagtctggggctgaggttaagaagcctggggcttcagtgaaggtgtcctgcaagggttctggctacaccttcaccagctactggatgcattgggtgaggcaggcgcctggccaacgtctagagtggatcggagagattgatccttctgagagtaatactaactacaatcaaaaattcaagggacgcgtcacattgactgtagacatttccgctagcacagcctacatggagctctccagcctgagatctgaggacactgcggtctactattgtgcaagagggggttacgacggatgggactatgctattgactactggggtcaaggcaccctggtcaccgtcagctcagcctccaccaagggcccatcggtcttccccctggcaccctcctccaagagcacctctgggggcacagcggccctgggctgcctggtcaaggactacttccccgaaccggtgacggtgtcgtggaactcaggcgccctgaccagcggcgtgcacaccttcccggctgtcctacagtcctcaggactctactccctcagcagcgtggtgaccgtgccctccagcagcttgggcacccagacctacatctgcaacgtgaatcacaagcccagcaacaccaaggtggacaagaaagttgagcccaaatcttgtgacaaaactcacacatgcccaccgtgcccagcacctgaactcgcgggggcaccgtcagtcttcctcttccccccaaaacccaaggacaccctcatgatctcccggacccctgaggtcacatgcgtggtggtggacgtgagccacgaagaccctgaggtcaagttcaactggtacgtggacggcgtggaggtgcataatgccaagacaaagccgcgggaggagcagtacaacagcacgtaccgtgtggtcagcgtcctcaccgtcctgcaccaggactggctgaatggcaaggagtacaagtgcaaggtctccaacaaagccctcccagcccccatcgagaaaaccatctccaaagccaaagggcagccccgagaaccacaggtgtacaccctgcccccatcccgggatgagctgaccaagaaccaggtcagcctgacctgcctggtcaaaggcttctatcccagcgacatcgccgtggagtgggagagcaatgggcagccggagaacaactacaagaccacgcctcccgtgctggactccgacggctccttcttcctctacagcaagctcaccgtggacaagagcaggtggcagcaggggaacgtcttctcatgctccgtgatgcatgaggctctgcacaaccactacacgcagaagagcctctccctgtctccgggtaaa

SEQ ID NO: 15 - DNA, 1448 bp, Artificial Sequence
  Description of Artificial Sequence: Synthetic polynucleotide
ggtaccagaattcctcaccatgggctggtcctgcatcatcctgtttctggtggccacagccacaggggtgcacagccaggtgcagctggtgcagtctggggctgaggtgaagaagccaggggcctctgtgaaggtgtcctgcaagggctctggctacaccttcaccagctactggatgcactgggtgcgccaggccccaggccagaggctggagtggatcggggagatcgacccctctgagagcaacaccaactacaaccagaagttcaagggcagggtgaccctgacagtggacatctctgccagcacagcctacatggagctgtccagcctgagatctgaggacacagctgtgtactactgtgccagggggggatatgatggctgggactatgccatcgactactggggccagggcaccctggtgacagtcagctcagccagcaccaagggcccctctgtgttccccctggcccccagcagcaagagcacctctgggggcacagctgccctgggctgcctggtgaaggactacttcccagagccagtgacagtgtcctggaactctggggccctgacatctggggtgcacaccttccctgctgtgctgcagtcctctggcctgtatagcctgtcctctgtggtgacagtgcccagcagcagcctgggcacccagacctacatctgcaatgtgaaccacaagcccagcaacacaaaggtggacaagaaggtggagcccaagagctgtgacaagacccacacctgccccccctgcccagccccagagctggctggggctccatctgtgtttctgttcccccccaagcccaaggacaccctgatgatcagcaggaccccagaggtgacctgtgtggtggtggatgtgagccatgaggatccagaggtgaagttcaattggtatgtggatggggtggaggtgcacaatgccaagaccaagcccagagaggagcagtacaacagcacctacagggtggtgtctgtgctgacagtgctgcaccaggactggctgaatggcaaggagtacaagtgcaaggtctccaataaggccctgccagcccccatcgaaaagaccatcagcaaggccaagggccagccaagggagccccaggtgtacaccctgcccccctccagagatgagctgaccaagaaccaggtgtccctgacctgtctggtgaagggcttctacccctctgacatcgctgtggagtgggagagcaatggccagccagagaacaactacaagaccacccccccagtgctggattctgatggcagcttcttcctgtacagcaagctgacagtggataagtccaggtggcagcagggcaatgtgttcagctgctctgtgatgcatgaggccctgcacaaccactacacccagaagagcctgtccctgagcccaggcaagtgatagtctagaggagctc

SEQ ID NO: 16 - DNA, 754 bp, Artificial Sequence
  Description of Artificial Sequence: Synthetic polynucleotide
ggtaccagcggccgcctcaccatgggctggtcctgcatcatcctgtttctggtggccacagccacaggggtgcactctgatgtggtgatgacccagagccccctgagcctgccagtgaccccaggggagccagccagcatcagctgcaggtccagccagagcctggccaagagctatggcaacacctacctgagctggtatctgcagaagccaggccagtccccccagctgctgatctatggcatcagcaacaggttctctggggtgccagacagattctctggctctgggtctggcacagacttcaccctgaagatcagcagggtggaggctgaggatgtgggggtgtactactgcctgcagggcacacaccagccctacacctttggccagggcaccaaggtggagatcaagcgtacggtggctgccccctctgtgttcatcttccccccctctgatgagcagctgaagtctgggacagcctctgtggtgtgcctgctgaacaacttctaccccagggaggccaaggtgcagtggaaggtggacaatgccctgcagtctggcaacagccaggagtctgtgacagagcaggacagcaaggactccacctacagcctgagcagcaccctgaccctgagcaaggctgactatgagaagcacaaggtgtacgcctgtgaggtgacccaccagggcctgtccagcccagtgaccaagagcttcaacaggggggagtgctgatagtctagaggagctc

SEQ ID NO: 17 - DNA, 1447 bp, Artificial Sequence
  Description of Artificial Sequence: Synthetic polynucleotide
ggtaccgaattcctcaccatgggctggtcctgcatcatcctgtttctggtggccaccgccaccggcgtgcacagccaggtgcagctggtgcagagcggagccgaggtgaagaagccaggcgccagcgtcaaggtgtcctgcaagggcagcggctacaccttcaccagctactggatgcactgggtgcggcaggccccaggccagaggctggagtggatcggcgagatcgaccccagcgagagcaacaccaactacaaccagaagttcaagggcagggtcaccctgaccgtggacatcagcgccagcaccgcctacatggagctgtccagcctgagaagcgaggacaccgccgtgtactactgcgccaggggcggctacgacggctgggactacgccatcgactactggggccagggcaccctggtgaccgtcagctcagccagcaccaagggccccagcgtgttccccctggcccccagcagcaagagcaccagcggcggcacagccgccctgggctgcctggtgaaggactacttccccgagcccgtgaccgtgtcctggaacagcggagccctgaccagcggggtgcacaccttccccgccgtgctgcagagcagcggcctgtacagcctgtccagcgtggtgacagtgcccagcagcagcctgggcacccagacctacatctgcaacgtgaaccacaagccctccaacaccaaggtggacaagaaggtggagcccaagagctgcgacaagacccacacctgccccccctgcccagcccccgagctggccggagccccctccgtgttcctgttcccccccaagcccaaggacaccctgatgatcagcaggacccccgaggtgacctgcgtggtggtggacgtgagccacgaggacccagaggtgaagttcaactggtacgtggacggcgtggaggtgcacaacgccaagaccaagcccagagaggagcagtacaacagcacctacagggtggtgtccgtgctgaccgtgctgcaccaggactggctgaacggcaaggaatacaagtgcaaggtctccaacaaggccctgcctgcccccatcgaaaagaccatcagcaaggccaagggccagccacgggagccccaggtgtacaccctgcccccctcccgggacgagctgaccaagaaccaggtgtccctgacctgtctggtgaagggcttctaccccagcgacatcgccgtggagtgggagagcaacggccagcccgagaacaactacaagaccacccccccagtgctggacagcgacggcagcttcttcctgtacagcaagctgacagtggacaagagcaggtggcagcagggcaacgtgttcagctgcagcgtgatgcacgaggccctgcacaaccactacacccagaagagcctgagcctgtcccccggcaagtgatagtctagaggagctc

SEQ ID NO: 18 - DNA, 753 bp, Artificial Sequence
  Description of Artificial Sequence: Synthetic polynucleotide
ggtaccgcggccgcctcaccatgggctggtcctgcatcatcctgtttctggtggccaccgccaccggcgtgcacagcgacgtggtgatgacccagagccccctgagcctgcccgtgaccccaggcgagcccgccagcatcagctgcaggtccagccagagcctggccaagagctacggcaacacctacctgagctggtatctgcagaagcccggccagtccccccagctgctgatctacggcatcagcaacaggttcagcggcgtgcccgacaggttctccggcagcggctccggcaccgacttcaccctgaaaatcagcagggtggaggccgaggacgtgggcgtgtactactgcctgcagggcacacaccagccctacaccttcggccagggcaccaaggtggaaatcaagcgtacggtggccgctcccagcgtgttcatcttcccccccagcgacgagcagctgaagagcggcaccgccagcgtggtgtgcctgctgaacaacttctacccccgggaggccaaggtgcagtggaaggtggacaacgccctgcagagcggcaacagccaggagagcgtcaccgagcaggacagcaaggactccacctacagcctgagcagcaccctgaccctgagcaaggccgactacgagaagcacaaggtgtacgcctgcgaggtgacccaccagggcctgtccagccccgtgaccaagagcttcaacaggggcgagtgctgatagtctagaggagctc

SEQ ID NO: 19 - DNA, 733 bp, Artificial Sequence
  Description of Artificial Sequence: Synthetic polynucleotide
atgggctggtcctgcatcatcctgtttctggtggccacmgccacmggsgtgcacwsygaygtggtgatgacccagagccccctgagcctgccmgtgaccccaggsgagccmgccagcatcagctgcaggtccaggcagagcctggccaagagctayggcaacacctacctgagccggtatctgcagaagccmggccagtcgccccagctgctgatctayggcatcagcaacaggttcwsyggsgtgccmgacagrttctcyggcwsyggstcyggcacmgacttcaccctgaaratcagcagggtggaggcygaggaygtgggsgtgtactactgcctgcagggcacacaccagccctacaccttyggccagggcaccaaggtggaratcaagcgtacggtggcygcycccwsygtgttcatcttcccccccwsygaygagcagctgaagwsyggsacmgccwsygtggtgtgcctgctgaacaacttctaccccmgggaggccaaggtgcagtggaaggtggacaaygccctgcagwsyggcaacagccaggagwsygtsacmgagcaggacagcaaggactccacctacagcctgagcagcaccctgaccctgagcaaggcygactaygagaagcacaaggtgtacgcctgygaggtgacccaccagggcctgtccagcccmgtgaccaagagcttcaacaggggsgagtgctgatagtctagaggagctc

SEQ ID NO: 20 - DNA, 1429 bp, Artificial Sequence
  Description of Artificial Sequence: Synthetic polynucleotide
atgggctggtcctgcatcatcctgtttctggtggccacmgccacmggsgtgcacagccaggtgcagctggtgcagwsyggrgcygaggtgaagaagccaggsgccwsygtsaaggtgtcctgcaagggcwsyggctacaccttcaccagctactggatgcactgggtgcgscaggccccaggccagaggctggagtggatcggsgagatcgaccccwsygagagcaacaccaactacaaccagaagttcaagggcagggtsaccctgacmgtggacatcwsygccagcacmgcctacatggagctgtccagcctgagawsygaggacacmgcygtgtactactgygccaggggsggmtaygayggctgggactaygccatcgactactggggccagggcaccctggtgacmgtcagctcagccagcaccaagggccccwsygtgttccccctggcccccagcagcaagagcaccwsyggsggcacagcygccctgggctgcctggtgaaggactacttcccmgagccmgtgacmgtgtcctggaacwsyggrgccctgacmwsyggggtgcacaccttcccygcygtgctgcagwscwsyggcctgtayagcctgtccwsygtggtgacagtgcccagcagcagcctgggcacccagacctacatctgcaaygtgaaccacaagcccwscaacacmaaggtggacaagaaggtggagcccaagagctgygacaagacccacacctgccccccctgcccagccccmgagctggcyggrgcyccmtcygtgttyctgttcccccccaagcccaaggacaccctgatgatcagcaggaccccmgaggtgacctgygtggtggtggaygtgagccaygaggayccagaggtgaagttcaaytggtaygtggayggsgtggaggtgcacaaygccaagaccaagcccagagaggagcagtacaacagcacctacagggtggtgtcygtgctgacmgtgctgcaccaggactggctgaayggcaaggartacaagtgcaaggtctccaayaaggccctgccwgcccccatcgaaaagaccatcagcaaggccaagggccagccamgggagccccaggtgtacaccctgcccccctccmgrgaygagctgaccaagaaccaggtgtccctgacctgtctggtgaagggcttctaccccwsygacatcgcygtggagtgggagagcaayggccagccmgagaacaactacaagaccacccccccagtgctggaywsygayggcagcttcttcctgtacagcaagctgacagtggayaagwscaggtggcagcagggcaaygtgttcagctgcwsygtgatgcaygaggccctgcacaaccactacacccagaagagcctgwscctgwscccmggcaagtgatagtctagaggagctc

SEQ ID NO: 21 - protein, 33 aa, Artificial Sequence
  Description of Artificial Sequence: Synthetic polypeptide
HGDGSFSDEMNTILDNLAARDFINWLIQTKITD

SEQ ID NO: 22 - protein, 121 aa, Artificial Sequence [sequence omitted]

SEQ ID NO: 23 - protein, 107 aa, Artificial Sequence [sequence omitted]

SEQ ID NO: 24 - protein, 7 aa, Artificial Sequence
  Description of Artificial Sequence: Synthetic peptide
GFTFDDY

SEQ ID NO: 25 - protein, 6 aa, Artificial Sequence
  Description of Artificial Sequence: Synthetic peptide
TWNSGH

SEQ ID NO: 26 - protein, 12 aa, Artificial Sequence
  Description of Artificial Sequence: Synthetic peptide
VSYLSTASSLDY

SEQ ID NO: 27 - protein, 8 aa, Artificial Sequence
  Description of Artificial Sequence: Synthetic peptide
QGIRNYLA

SEQ ID NO: 28 - protein, 7 aa, Artificial Sequence
  Description of Artificial Sequence: Synthetic peptide
AASTLQS

SEQ ID NO: 29 - protein, 9 aa, Artificial Sequence
  Description of Artificial Sequence: Synthetic peptide
QRYNRAPYT

SEQ ID NO: 30 - protein, 451 aa, Artificial Sequence
  Description of Artificial Sequence: Synthetic polypeptide
EVQLVESGGGLVQPGRSLRLSCAASGFTFDDYAMHWVRQAPGKGLEWVSAITWNSGHIDYADSVEGRFTISRDNAKNSLYLQMNSLRAEDTAVYYCAKVSYLSTASSLDYWGQGTLVTVSSASTKGPSVFPLAPSSKSTSGGTAALGCLVKDYFPEPVTVSWNSGALTSGVHTFPAVLQSSGLYSLSSVVTVPSSSLGTQTYICNVNHKPSNTKVDKKVEPKSCDKTHTCPPCPAPELLGGPSVFLFPPKPKDTLMISRTPEVTCVVVDVSHEDPEVKFNWYVDGVEVHNAKTKPREEQYNSTYRVVSVLTVLHQDWLNGKEYKCKVSNKALPAPIEKTISKAKGQPREPQVYTLPPSRDELTKNQVSLTCLVKGFYPSDIAVEWESNGQPENNYKTTPPVLDSDGSFFLYSKLTVDKSRWQQGNVFSCSVMHEALHNHYTQKSLSLSPGK

SEQ ID NO: 31 - protein, 214 aa, Artificial Sequence
  Description of Artificial Sequence: Synthetic polypeptide
DIQMTQSPSSLSASVGDRVTITCRASQGIRNYLAWYQQKPGKAPKLLIYAASTLQSGVPSRFSGSGSGTDFTLTISSLQPEDVATYYCQRYNRAPYTFGQGTKVEIKRTVAAPSVFIFPPSDEQLKSGTASVVCLLNNFYPREAKVQWKVDNALQSGNSQESVTEQDSKDSTYSLSSTLTLSKADYEKHKVYACEVTHQGLSSPVTKSFNRGEC

SEQ ID NO: 32 - protein, 119 aa, Artificial Sequence
  Description of Artificial Sequence: Synthetic polypeptide
EVQLVQSGAEVKKPGESLKISCKGSGYSFTTYWLGWVRQMPGKGLDWIGIMSPVDSDIRYSPSFQGQVTMSVDKSITTAYLQWNSLKASDTAMYYCARRRPGQGYFDFWGQGTLVTVSS

SEQ ID NO: 33 - protein, 107 aa, Artificial Sequence
  Description of Artificial Sequence: Synthetic polypeptide
DIQMTQSPSSLSASVGDRVTITCRASQGISSWLAWYQQKPEKAPKSLIYAASSLQSGVPSRFSGSGSGTDFTLTISSLQPEDFATYYCQQYNIYPYTFGQGTKLEIK

SEQ ID NO: 34 - protein, 7 aa, Artificial Sequence
  Description of Artificial Sequence: Synthetic peptide
GYSFTTY

SEQ ID NO: 35 - protein, 6 aa, Artificial Sequence
  Description of Artificial Sequence: Synthetic peptide
SPVDSD

SEQ ID NO: 36 - protein, 10 aa, Artificial Sequence
  Description of Artificial Sequence: Synthetic peptide
RRPGQGYFDF

SEQ ID NO: 37 - protein, 8 aa, Artificial Sequence
  Description of Artificial Sequence: Synthetic peptide
QGISSWLA

SEQ ID NO: 38 - protein, 7 aa, Artificial Sequence
  Description of Artificial Sequence: Synthetic peptide
AASSLQS

SEQ ID NO: 39 - protein, 9 aa, Artificial Sequence
  Description of Artificial Sequence: Synthetic peptide
QQYNIYPYT

SEQ ID NO: 40 - protein, 449 aa, Artificial Sequence
  Description of Artificial Sequence: Synthetic polypeptide
EVQLVQSGAEVKKPGESLKISCKGSGYSFTTYWLGWVRQMPGKGLDWIGIMSPVDSDIRYSPSFQGQVTMSVDKSITTAYLQWNSLKASDTAMYYCARRRPGQGYFDFWGQGTLVTVSSSSTKGPSVFPLAPSSKSTSGGTAALGCLVKDYFPEPVTVSWNSGALTSGVHTFPAVLQSSGLYSLSSVVTVPSSSLGTQTYICNVNHKPSNTKVDKRVEPKSCDKTHTCPPCPAPELLGGPSVFLFPPKPKDTLMISRTPEVTCVVVDVSHEDPEVKFNWYVDGVEVHNAKTKPREEQYNSTYRVVSVLTVLHQDWLNGKEYKCKVSNKALPAPIEKTISKAKGQPREPQVYTLPPSRDELTKNQVSLTCLVKGFYPSDIAVEWESNGQPENNYKTTPPVLDSDGSFFLYSKLTVDKSRWQQGNVFSCSVMHEALHNHYTQKSLSLSPGK

SEQ ID NO: 41 - protein, 214 aa, Artificial Sequence
  Description of Artificial Sequence: Synthetic polypeptide
DIQMTQSPSSLSASVGDRVTITCRASQGISSWLAWYQQKPEKAPKSLIYAASSLQSGVPSRFSGSGSGTDFTLTISSLQPEDFATYYCQQYNIYPYTFGQGTKLEIKRTVAAPSVFIFPPSDEQLKSGTASVVCLLNNFYPREAKVQWKVDNALQSGNSQESVTEQDSKDSTYSLSSTLTLSKADYEKHKVYACEVTHQGLSSPVTKSFNRGEC

SEQ ID NO: 42 - DNA, 363 bp, Artificial Sequence
  Description of Artificial Sequence: Synthetic polynucleotide
gaggtgcagctggtggagagcggcggcggcctggtgcagcccggccggagcctgcggctgagctgcgccgccagcggcttcaccttcgacgactacgccatgcactgggtgcggcaggcccccggcaagggcctggagtgggtgagcgccatcacctggaacagcggccacatcgactacgccgacagcgtggagggccggttcaccatcagccgggacaacgccaagaacagcctgtacctgcagatgaacagcctgcgggccgaggacaccgccgtgtactactgcgccaaggtgagctacctgagcaccgccagcagcctggactactggggccagggcaccctggtgaccgtgagcagc

SEQ ID NO: 43 - DNA, 321 bp, Artificial Sequence
  Description of Artificial Sequence: Synthetic polynucleotide
gacatccagatgacccagagccccagcagcctgagcgccagcgtgggcgaccgggtgaccatcacctgccgggccagccagggcatccggaactacctggcctggtaccagcagaagcccggcaaggcccccaagctgctgatctacgccgccagcaccctgcagagcggcgtgcccagccggttcagcggcagcggcagcggcaccgacttcaccctgaccatcagcagcctgcagcccgaggacgtggccacctactactgccagcggtacaaccgggccccctacaccttcggccagggcaccaaggtggagatcaag

SEQ ID NO: 44 - DNA, 1353 bp, Artificial Sequence
  Description of Artificial Sequence: Synthetic polynucleotide
gaggtgcagctggtggagagcggcggcggcctggtgcagcccggccggagcctgcggctgagctgcgccgccagcggcttcaccttcgacgactacgccatgcactgggtgcggcaggcccccggcaagggcctggagtgggtgagcgccatcacctggaacagcggccacatcgactacgccgacagcgtggagggccggttcaccatcagccgggacaacgccaagaacagcctgtacctgcagatgaacagcctgcgggccgaggacaccgccgtgtactactgcgccaaggtgagctacctgagcaccgccagcagcctggactactggggccagggcaccctggtgaccgtgagcagcgccagcaccaagggccccagcgtgttccccctggcccccagcagcaagagcaccagcggcggcaccgccgccctgggctgcctggtgaaggactacttccccgagcccgtgaccgtgagctggaacagcggcgccctgaccagcggcgtgcacaccttccccgccgtgctgcagagcagcggcctgtacagcctgagcagcgtggtgaccgtgcccagcagcagcctgggcacccagacctacatctgcaacgtgaaccacaagcccagcaacaccaaggtggacaagaaggtggagcccaagagctgcgacaagacccacacctgccccccctgccccgcccccgagctgctgggcggccccagcgtgttcctgttcccccccaagcccaaggacaccctgatgatcagccggacccccgaggtgacctgcgtggtggtggacgtgagccacgaggaccccgaggtgaagttcaactggtacgtggacggcgtggaggtgcacaacgccaagaccaagccccgggaggagcagtacaacagcacctaccgggtggtgagcgtgctgaccgtgctgcaccaggactggctgaacggcaaggagtacaagtgcaaggtgagcaacaaggccctgcccgcccccatcgagaagaccatcagcaaggccaagggccagccccgggagccccaggtgtacaccctgccccccagccgggacgagctgaccaagaaccaggtgagcctgacctgcctggtgaagggcttctaccccagcgacatcgccgtggagtgggagagcaacggccagcccgagaacaactacaagaccaccccccccgtgctggacagcgacggcagcttcttcctgtacagcaagctgaccgtggacaagagccggtggcagcagggcaacgtgttcagctgcagcgtgatgcacgaggccctgcacaaccactacacccagaagagcctgagcctgagccccggcaag

SEQ ID NO: 45 - DNA, 642 bp, Artificial Sequence
  Description of Artificial Sequence: Synthetic polynucleotide
gacatccagatgacccagagccccagcagcctgagcgccagcgtgggcgaccgggtgaccatcacctgccgggccagccagggcatccggaactacctggcctggtaccagcagaagcccggcaaggcccccaagctgctgatctacgccgccagcaccctgcagagcggcgtgcccagccggttcagcggcagcggcagcggcaccgacttcaccctgaccatcagcagcctgcagcccgaggacgtggccacctactactgccagcggtacaaccgggccccctacaccttcggccagggcaccaaggtggagatcaagcggaccgtggccgcccccagcgtgttcatcttcccccccagcgacgagcagctgaagagcggcaccgccagcgtggtgtgcctgctgaacaacttctacccccgggaggccaaggtgcagtggaaggtggacaacgccctgcagagcggcaacagccaggagagcgtgaccgagcaggacagcaaggacagcacctacagcctgagcagcaccctgaccctgagcaaggccgactacgagaagcacaaggtgtacgcctgcgaggtgacccaccagggcctgagcagccccgtgaccaagagcttcaaccggggcgagtgc

SEQ ID NO: 46 - DNA, 357 bp, Artificial Sequence
  Description of Artificial Sequence: Synthetic polynucleotide
gaggtgcagctggtgcagagcggcgccgaggtgaagaagcccggcgagagcctgaagatcagctgcaagggcagcggctacagcttcaccacctactggctgggctgggtgcggcagatgcccggcaagggcctggactggatcggcatcatgagccccgtggacagcgacatccggtacagccccagcttccagggccaggtgaccatgagcgtggacaagagcatcaccaccgcctacctgcagtggaacagcctgaaggccagcgacaccgccatgtactactgcgcccggcggcggcccggccagggctacttcgacttctggggccagggcaccctggtgaccgtgagcagc

SEQ ID NO: 47 - DNA, 321 bp, Artificial Sequence
  Description of Artificial Sequence: Synthetic polynucleotide
gacatccagatgacccagagccccagcagcctgagcgccagcgtgggcgaccgggtgaccatcacctgccgggccagccagggcatcagcagctggctggcctggtaccagcagaagcccgagaaggcccccaagagcctgatctacgccgccagcagcctgcagagcggcgtgcccagccggttcagcggcagcggcagcggcaccgacttcaccctgaccatcagcagcctgcagcccgaggacttcgccacctactactgccagcagtacaacatctacccctacaccttcggccagggcaccaagctggagatcaag

SEQ ID NO: 48 - DNA, 1347 bp, Artificial Sequence
  Description of Artificial Sequence: Synthetic polynucleotide
gaggtgcagctggtgcagagcggcgccgaggtgaagaagcccggcgagagcctgaagatcagctgcaagggcagcggctacagcttcaccacctactggctgggctgggtgcggcagatgcccggcaagggcctggactggatcggcatcatgagccccgtggacagcgacatccggtacagccccagcttccagggccaggtgaccatgagcgtggacaagagcatcaccaccgcctacctgcagtggaacagcctgaaggccagcgacaccgccatgtactactgcgcccggcggcggcccggccagggctacttcgacttctggggccagggcaccctggtgaccgtgagcagcagcagcaccaagggccccagcgtgttccccctggcccccagcagcaagagcaccagcggcggcaccgccgccctgggctgcctggtgaaggactacttccccgagcccgtgaccgtgagctggaacagcggcgccctgaccagcggcgtgcacaccttccccgccgtgctgcagagcagcggcctgtacagcctgagcagcgtggtgaccgtgcccagcagcagcctgggcacccagacctacatctgcaacgtgaaccacaagcccagcaacaccaaggtggacaagcgggtggagcccaagagctgcgacaagacccacacctgccccccctgccccgcccccgagctgctgggcggccccagcgtgttcctgttcccccccaagcccaaggacaccctgatgatcagccggacccccgaggtgacctgcgtggtggtggacgtgagccacgaggaccccgaggtgaagttcaactggtacgtggacggcgtggaggtgcacaacgccaagaccaagccccgggaggagcagtacaacagcacctaccgggtggtgagcgtgctgaccgtgctgcaccaggactggctgaacggcaaggagtacaagtgcaaggtgagcaacaaggccctgcccgcccccatcgagaagaccatcagcaaggccaagggccagccccgggagccccaggtgtacaccctgccccccagccgggacgagctgaccaagaaccaggtgagcctgacctgcctggtgaagggcttctaccccagcgacatcgccgtggagtgggagagcaacggccagcccgagaacaactacaagaccaccccccccgtgctggacagcgacggcagcttcttcctgtacagcaagctgaccgtggacaagagccggtggcagcagggcaacgtgttcagctgcagcgtgatgcacgaggccctgcacaaccactacacccagaagagcctgagcctgagccccggcaag

SEQ ID NO: 49 - DNA, 642 bp, Artificial Sequence
  Description of Artificial Sequence: Synthetic polynucleotide
gacatccagatgacccagagccccagcagcctgagcgccagcgtgggcgaccgggtgaccatcacctgccgggccagccagggcatcagcagctggctggcctggtaccagcagaagcccgagaaggcccccaagagcctgatctacgccgccagcagcctgcagagcggcgtgcccagccggttcagcggcagcggcagcggcaccgacttcaccctgaccatcagcagcctgcagcccgaggacttcgccacctactactgccagcagtacaacatctacccctacaccttcggccagggcaccaagctggagatcaagcggaccgtggccgcccccagcgtgttcatcttcccccccagcgacgagcagctgaagagcggcaccgccagcgtggtgtgcctgctgaacaacttctacccccgggaggccaaggtgcagtggaaggtggacaacgccctgcagagcggcaacagccaggagagcgtgaccgagcaggacagcaaggacagcacctacagcctgagcagcaccctgaccctgagcaaggccgactacgagaagcacaaggtgtacgcctgcgaggtgacccaccagggcctgagcagccccgtgaccaagagcttcaaccggggcgagtgc

SEQ ID NO: 50 - protein, 628 aa, Artificial Sequence
  Description of Artificial Sequence: Synthetic polypeptide
AEAPHLVHVDAARALWPLRRFWRSTGFCPPLPHSQADQYVLSWDQQLNLAYVGAVPHRGIKQVRTHWLLELVTTRGSTGRGLSYNFTHLDGYLDLLRENQLLPGFELMGSASGHFTDFEDKQQVFEWKDLVSSLARRYIGRYGLAHVSKWNFETWNEPDHHDFDNVSMTMQGFLNYYDACSEGLRAASPALRLGGPGDSFHTPPRSPLSWGLLRHCHDGTNFFTGEAGVRLDYISLHRKGARSSISILEQEKVVAQQIRQLFPKFADTPIYNDEADPLVGWSLPQPWRADVTYAAMVVKVIAQHQNLLLANTTSAFPYALLSNDNAFLSYHPHPFAQRTLTARFQVNNTRPPHVQLLRKPVLTAMGLLALLDEEQLWAEVSQAGTVLDSNHTVGVLASAHRPQGPADAWRAAVLIYASDDTRAHPNRSVAVTLRLRGVPPGPGLVYVTRYLDNGLCSPDGEWRRLGRPVFPTAEQFRRMRAAEDPVAAAPRPLPAGGRLTLRPALRLPSLLLVHVCARPEKPPGQVTRLRALPLTQGQLVLVWSDEHVGSKCLWTYEIQFSQDGKAYTPVSRKPSTFNLFVFSPDTGAVSGSYRVRALDYWARPGPFSDPVPYLEVPVPRGPPSPGNP

SEQ ID NO: 51 - protein, 525 aa, Artificial Sequence
  Description of Artificial Sequence: Synthetic polypeptide
SETQANSTTDALNVLLIIVDDLRPSLGCYGDKLVRSPNIDQLASHSLLFQNAFAQQAVCAPSRVSFLTGRRPDTTRLYDFNSYWRVHAGNFSTIPQYFKENGYVTMSVGKVFHPGISSNHTDDSPYSWSFPPYHPSSEKYENTKTCRGPDGELHANLLCPVDVLDVPEGTLPDKQSTEQAIQLLEKMKTSASPFFLAVGYHKPHIPFRYPKEFQKLYPLENITLAPDPEVPDGLPPVAYNPWMDIRQREDVQALNISVPYGPIPVDFQRKIRQSYFASVSYLDTQVGRLLSALDDLQLANSTIIAFTSDHGWALGEHGEWAKYSNFDVATHVPLIFYVPGRTASLPEAGEKLFPYLDPFDSASQLMEPGRQSMDLVELVSLFPTLAGLAGLQVPPRCPVPSFHVELCREGKNLLKHFRFRDLEEDPYLPGNPRELIAYSQYPRPSDIPQWNSDKPSLKDIKIMGYSIRTIDYRYTVWVGFNPDEFLANFSDIHAGELYFVDSDPLQDHNMYNDSQGGDLFQLLMP

SEQ ID NO: 52 - protein, 509 aa, Homo sapiens
MSMGAPRSLLLALAAGLAVARPPNIVLIFADDLGYGDLGCYGHPSSTTPNLDQLAAGGLRFTDFYVPVSLCTPSRAALLTGRLPVRMGMYPGVLVPSSRGGLPLEEVTVAEVLAARGYLTGMAGKWHLGVGPEGAFLPPHQGFHRFLGIPYSHDQGPCQNLTCFPPATPCDGGCDQGLVPIPLLANLSVEAQPPWLPGLEARYMAFAHDLMADAQRQDRPFFLYYASHHTHYPQFSGQSFAERSGRGPFGDSLMELDAAVGTLMTAIGDLGLLEETLVIFTADNGPETMRMSRGGCSGLLRCGKGTTYEGGVREPALAFWPGHIAPGVTHELASSLDLLPTLAALAGAPLPNVTLDGFDLSPLLLGTGKSPRQSLFFYPSYPDEVRGVFAVRTGKYKAHFFTQGSAHSDTTADPACHASSSLTAHEPPLLYDLSKDPGENYNLLGGVAGATPEVLQALKQLQLLKAQLDAAVTFGPSQVARGEDPALQICCHPGCTPRPACCHCPDPHA